European Patent Application EP 4 707 279 A1, published March 11, 2026. Title: 新型コロナウイルス感染症の処置または予防用医薬としての置換三環式複素環化合物. Applicant: 大分大学. Application WO. The sequence listing filed with the application follows.

SEQUENCE LISTING (3 sequences)

SEQ ID NO: 1 - DNA, 20 bp, synthetic construct
  source 1..20: mol_type = other DNA
cgcatacagtcttrcaggct

SEQ ID NO: 2 - DNA, 24 bp, synthetic construct
  source 1..24: mol_type = other DNA
gtgtgatgttgawatgacatggtc

SEQ ID NO: 3 - DNA, 26 bp, synthetic construct
  source 1..26: mol_type = other DNA
ttaagatgtggcttgcatacgtagac